European Patent Specification EP 3 802 877 B1, published November 5, 2025. Title: METHOD. Applicant: Oxford Nanopore Technologies Limited. The sequence listing filed with the application follows.

SEQUENCE LISTING (53 sequences)

SEQ ID NO: 1 - DNA, 40 bp, Artificial Sequence
  Control Adapter NB01 (barcode top strand)
aaggttaacacaaagacaccgacaactttcttcagcacct

SEQ ID NO: 2 - DNA, 45 bp, Artificial Sequence
  Control adapter NB01 (barcode bottom strand)
ggtgctgaagaaagttgtcggtgtctttgtgttaaccttagcaat

SEQ ID NO: 3 - DNA, 59 bp, Artificial Sequence
  Follow-On Adapter (barcode top strand)
ggcgtctgcttgggtgtttaacctttttgtcagagaggttccaagtcagagaggttcct

SEQ ID NO: 4 - DNA, 64 bp, Artificial Sequence
  Follow-On Adapter (barcode bottom strand)
ggaacctctctgacttggaacctctctgacaaaaaggttaaacacccaagcagacgccagcaat

SEQ ID NO: 5 - DNA, 59 bp, Artificial Sequence; identical to SEQ ID NO: 3
  Follow-On Adapter (barcode top strand)
  misc_binding (23)..(24): nucleotides separated by 4x iSp18

SEQ ID NO: 6 - DNA, 64 bp, Artificial Sequence; identical to SEQ ID NO: 4
  Follow-On Adapter (barcode bottom strand)
  misc_binding (35)..(36): nucleotides separated by 4x iSp18

SEQ ID NO: 7 - protein, 262 aa, Escherichia coli
CLTAPPKEAARPTLMPRAQSYKDLTHLPAPTGKIFVSVYNIQDETGQFKPYPASNFSTAVPQSATAMLVTALKDSRWFIPLERQGLQNLLNERKIIRAAQENGTVAINNRIPLQSLTAANIMVEGSIIGYESNVKSGGVGARYFGIGADTQYQLDQIAVNLRVVNVSTGEILSSVNTSKTILSYEVQAGVFRFIDYQRLLEGEVGYTSNEPVMLCLMSAIETGVIFLINDGIDRGLWDLQNKAERQNDILVKYRHMSVPPES

SEQ ID NO: 8 - DNA, 16 bp, Artificial Sequence
  Morpholino oligo
ggaacctctctgacaa

SEQ ID NO: 9 - DNA, 17 bp, Artificial Sequence
  Tether
  misc_binding (2)..(3): nucleotides separated by 4x iSp18
ttttgaccgctcgcctc

SEQ ID NO: 10 - DNA, 12068 bp, Artificial Sequence
  Basecall_Alignment_template 90e5fe72_read_ch2_file10
tggtttgtcagagaggttcaagtccagggttccttgcctgtcatctatcttcggcgtctgcttgggtgttaacgcctctgcaccggacggtcccctcgcccctttgaggagggttaggaagagaaaaccgcacctgtaccggatcggttatttcgcattcttatcagacccactgcaaccgctgaatatgcaggcataacaggtgcaggatcaccaggcaatgcagcaggtaaatatcattgccgtcccagactttggtggtgaccttattgtccacgtccagctcctgccaccgggaaccatttcatagtccatccaggtacttatgcagtactctcccaccatgtttgataccaggtttccttggcgatcgccagtattgacggtgtaaacgcgtaggccgtacccattgcttcgacgataggccagcgtacacgttcgcggaccaccggtttccttcccagtcaacgacataaacggctccgtccgcgccatcggtgcccaggcatcgcgcacggtggcgttaaacgaacctttggcatcttctagcaacctgctggtggttgttcgcaacgggcttcccagggccatatggatgtacggcggcattaaacggccccattcgatccggtggcctggtgcactcgggcgcgcggaagcgatgcgccgggttatctttgttgtaatcccggcagccggattccactgggtatcagtgttcgtgctgcccgataatgattatttctggcgacatcgtggatgtcacggaagccacgcgaatcgcgcgatcagccattttgtcggtgacgtcataaacaatcgaagcttccaccgcgtgcatattggcattgccgccgcggtactcttcgattttctgaaggcttcgtcccgggattcaggcatatcttcttctccagaaatatttctcgataatttcgtatgggccttaatcagtagcgcgcttccaggtgaccgtttggcgacggcgctggcggcacccagcggaaacaaagtgttagtaagccctgttgcaggcatccaccacgccctctgatgccgttcgcacgcggcgtaccagccgccataattttatccgcaccatcgccgttcatggctttgatgccgtgatcaaccaacgatggcgccaggtcagcccatcgccgcaaccagcgatcgcgtgcaacatacgagcggtgatccacagatgggtgcccatctcttctttgatttgccctttgtgcctaaccagccatgcagtcggcactacggaattttaccaaaatcaaagatgcggtcggtttcctgttcagccaacggttggcagcagggtgttaaaccatttcattcataccatctcatcttggcggcgtttagccatcatttcgtcgacgatatcgccaagttgttgtaatttctgattacaaacgtcacgcagcatcagctcgttgtctggtaaaccgacgaccgtcttgaactgcacggcctgccaggaatccccgataacccaccgtcgttactgccacgcgtacgacgcaggaacgatttttcgtcgacaccgaagagatctcacccatggcgccattaatgctgtcattcagacgttgtgaagcacagaaagctcttgttgcggacctttgccataaagcggcattttcagctttgtgaaggtcagcgccactttctcgcccggctctttgagcacggcatcgatgatcagcaaccgcgatcgaatttatgctcacggcacaacggtgggcggacgctggttcgtgatgcttaccagaccgtgagtggcacagttcgttgaactctttcaccatatcgaagacgttgctgcgcatcttcatcactacgccacagcaccagcagttttaggctttgccaccgtcttgtttgatcttgtggattgattttgcggtcagcaaccacgctatcgtggagattcgttctgggaatgaactttcatcggcggcgaccgcaatcatggcgcaactttgtaatcgcattttgctcaaccacctggcggtaaccgtgacgatctaccaagtccttgagcataaggcgaagacgcgccgccggcgttaacacgaaatccagttaaaacgctactcctgagcttctggaagggcggtgccccagccgcggcaaacatcatgcacgctaaacttctgcgctgatcgacctgctgcgtagcaaaaccgccgatgcgcgtaatgtcgttgatggtgtgcttattcattcatttattccttttatccgatcgttacattttactttggcagtcatcccagcgcgacacggacctgttcaagaatggcggaccgatctggcgacccgcgacccgctgcgcgcctggctataaacctcccatcgggcagcccagcggcattggcacatgcagctggttggcgacatcaagggcgatgcaagattcttctgggcaagatcgatcatgaaggcgggaaaagatctccgctgaggactttgtttggccaggaagtggtgaagtgacctttaccggcagcatttgctttcatcgcgacggcaacatcgaggaagttagggcttcgcacaaacggcaacttctgccgaaagcacgccaggcgcaatgcctcgccagttgttgatgagcaacgcggatccccatgcccggaccgccagcgttgatcaactcactgccgctcaccatcggatcggtgtggcacgtccaactgttcaacggtgccgccagccagccagtaacagagtaccggtaatggcatttgcagaagtacggcctaccggtgggtgtcatcatactgaaactgcggcaccatcggcaatcaattcggttttgcagcggatggatggtggacatatcaatgaccaacacatggtgataaagccttcgcaaaacgccgtttcaccgaacaacacgttgcgcaccagatcgccattcggcaacatggtatgataaattcggcatctttagcggcctgccggttggcggcggggtcacgctgtctaccagatactacaccttcggcgttcacatcaaagacgcgaagttgatgcccttgctgcaataaattgctcaccggtggcggaccatttgtcctaaaccgataaacgcgattgctgccgcaaccctcctcctagaatatggtgtgctcacttttgtcatttatgacatgctttgcttgtctgttttgatcgtatttgtaatttatcgtcaagattgacagccgtcaccccaaacaattggtgaggtggtagacgcatcccaaatcactgagaatgaccatgattcattgttgccaatggccaagtaccaaccgtgatggatcgcatctattacgtggaaggaataccgacggagagcgtgaaaccgtggcgaggtatactggagagttggtggcgggccagcggcgacggcggcggttgcggcagcaggctgcgaggcgcaaggtcatttattggtcacgtgggtgatggcggctggtggcaacctgctggcagagctggaatcctgggcgttaacacccgttacgcaaacgagcataaccaggcgaaatattgcaatcaccatcatggtggatacaaggcgagcggataatcattaactacccccatgccggatcctgctgcctgacagagtggttggagaattgatttctctccggtgggatgttggctggcagatgtacgctggcacgacgagcgctaaaagccttcgccctggccgtcaggcgggtgtgatgaccgttctggacggggacgatgcgccgcaggaccatccggtgaaactggtggcattaagcgatcacgcggcctttcagaaccggtctggcagcaacgggcgtgaagatggcttggtgcgctaaaacaggcacaaacgctctaaatggtcatgtctatgtgaccagggtagccgcgagctgcgatagctggaaaatggtgggcgtcgcatcgtagccttcaaagttgatgtggtagataccacaggtgcgggtgatgttttcacggcgcgcacagcggtggcactggctggcaacaagtggggatttagcgagtcggtccaactacgtaacagtgtggcaacgttaaaatacgtcggtggacgaccgggatctgactgtgatcaaacccgatctttgtcacttttgtatgaaatgccaggggtgatggtttcgaggaattttcgcaggccttaccgaactaaccggtaacccgcagcgaccaactcctcctgctgatcgccgagcgggtatatgaatattgatgagctggcaaatcgctggatgtctccacacagacggtccgcgggatattcgtagtcatgagcaggctgattacgcactgcagctcacggtggcgcggtcagctcgcatcagtgtgacgttcggcagcgtgaggtttcgcaagctcgagaaaaacgttgccgaagcggtggcgaactatattcctgatggttcaacaatatttatcaccagtggtacggcttctattcgacgtatttgcccaggcgttgccaaccataatcatttacggataatctaccagcttgaagcctcgtgtggcgcatattgctacaacccgcgctttgaagtggtgcccggcggtacgttgcgctctcgccaatggcgggatcattggccttccggcggcgtcgctgtggccgatttcgtgcgcgattatcggtaacaagcgttgccggccggtgagcgatggcgcgttgatggagtttgataagcagaaactaacggctgggtgaaaacgatgatggcgcacccgaaatattctggtcgccgatcacacaagtatcatgccttcggcagcggttgaaattgataacgtggcacaggtcactgcgctcttaccgacgagctgccgcccgctgcgctaaatcacgcttacaagacaataggtaaatcattcttccccaggagagacgcgcgttacgaccgttaacctggccataccttgccacaacccaaacccatcctttccactacagttaatttcttgtggcgcgaaagacacaaatactctatatctttgatttgagtaatgtgattatcaatgtcaacaccaacgtgtgctggggcctgggcgattgcgcatgttacttcagcatcgcttaagaagagtttattgctgggagcgtttcatctggcatgggcattgaaattagcgacaagcgttcacagagagcgctgtatgtctgaatggctctaccactaagctacgacagttctctcacggctggcgacagtgtttgttgcgctacgccggaagtgatcgccgtaatgcataaactacctgcgtgacaggggcatcgtggtggtgctttccaataccaacctgcataccaccttctagcccggaagaatacccgaaattcgtgatgctgctattatatctatctgtcgcagatctggggatgcgcaaacctgaagcacgaatttaccagcatgttttgcaggcggaaggttttcacccagcgatacggtctttcgacgataacgccgataatatgaagggcaatcaactgggcattaccggtgttcggtgaagataaaccaccatccaagctatttcgcagtgttatgtaaaaaccattcaggacaaaactaaggcaccatgccatccactattgggcctggcacaaaactactctggcagcacgtattgaggacaacatgacaacctggcggtaaccttgcctatgcatttatgctctcggctaattcgccgctggttgccgttgttttgcgcttttcgccgcttttcccatgttttccgacgtcagcattcagttacgtcactttattattttgtaactttctgcctgctgcagcgatgttattcagcggtatatgaacaatttgttgccaattcaacaagatgaccgccgttggggctgatgggctgatcgtcaccgcgttattgttgatgtactccatccgatagcgcgttgaataccatctggcgcagtaagtaagcgcgaccaaaatttactcgttcaccgtcactggtggattttaacactaaagacccgcttctggcaagggccagtctggcgatcagttcctgttgctctccctgcgctgggcgaaacgtctcgctctgtcatcgataacgtgcgtatttttcccgttgctgttgtcgtggatctctccttctggttgccagctggcattgttctaccatccgtacctaaccgcggcgcgattgtcagcgtttgtcgccacactcctgttcgaagcaggaaaggtttcgcgcatatctacatgttcccgtctatcagctcatttatggtgtgcggcggtgatccccattctttgtttgggtctactggacatggtgtatcgtcttcgcagcgccgaagtactgtcactctcgggaataccgcaaaagctaaaacaagcagcttcgacaagaagacgacgaaccatgattgcattaattcaacgcgtaacccgtgccagcgtcaccgtggagagaagtgggcgagggagtagctgggactttgcggtgttattagcggtgctcaaaggtgtgaacgaaagcaaaccatctgtgcgagcattaacagctaccgcatctttatgatgcgaggcagatgaatctccagcgatgcaacgggcggcggcagtgtgctggtggtttcccagtttaccctcgccaccagatattctgaacaggggatacttaagtttctctcaggtgcatcacggatcgcgcagggcgttatatgactatttcgtcgaacgctgccgtcggcaagagatgaacacaccgacaggccgcttcgctgcggatatgcaggtatctggtcagccggccagccccatgtgacattctgtgatttgcagtgctgagccagcttccggtttgtcacgggaaacgaaagtatcgctatgtatctgccaggttccacaaacagaagaagaattgagagcgttactatcagtttcgctggaaatgttgcgcccttcatcaacaggttcggaacacgcgcgtgggatgcgatggcgcatcgcagatggtcacgtcgacgacagggtaatctcggtaacggtaaactgcgactgtatattgtctaccgacaatgaagcgtccattcaacatggccgttcatcccggcgtgcgggacaagggttaggcgctgatggcgatgaccacaggtcggtggcgcgtcaggaagagcgttaagcgcatgactaacagcgcccgtgaagacgcggtgcggagttttcgccagcgggtttgtgtcagggagaaatcaccacataaccacgccgattcgccatttttgatgattaagcccgtcgcctcgttgacattcaccgcatcgcggcgactggtgcgcctggctgtgggcggtacgaacatatcgcgggtgaaaaatgggcgtgcgcattcagcaatataccgggcaaaatttatcactaccatgccgaaaccggcaatcaagtccgcaccatacgctgtttaccgaagacatttctcggcgacgctcactggactggggacttatctgtgatacgcgtgaacgccacctcggcgaacgattattcttgcggatacgcatatccacttcaaccagccgattggcggtaaacctcgtgcggtacgccgacctcggtatacgcaagcggcgatctcgaccgtcgcgcgcggacgaaagcaggtgcagatgcaggtcgaaatctttggcaacagggctaccgggtgcagtgtttgaaggcacgtatgtcgttctgcttgcccgcgaaagccatttggcccgtatgaaggcgggcgagtagctgatggaaggcgaacacctctctctcttcaggtgcattatgatagatcgccaagctatttcagttgctgtaaataagaactctataagttacgcattcttcttcgttggctccatgcggtgtcttgccacatcactgttcaggagcatttaaataatactttagcgaactggtggcaattatcacgccgaatagcgcttattccatcatcttagttcatgtttgagcgatttttgatagtcaaaaccccactctggtgccatacttttctcttaaatactttaaaatctatagctaacaaacaatatacaaagataatggatagctcgtcagtatcaaccatttaccctttcttgtgttatgaatattatgttgtatgtttgctcttaaaccgtgggaaggaggctataatggttgccaatataatctatttctgtgaaagttattctgttgttaatttgaaaacaactttcccagactgttaccaacaaaattatatgatgaacaagtaaagaccggttggtggcagtactacaaccgatgcgatgaagattaatttcaccgccaaatcctggtgctgttaggatgctggcgttttcggctacaccattcaagattatgcaaataatatctcagaccaacaatatattcttaacacccataattcatctgagcgatactaaaccattttgagtaataagtaaacagctacagcactcttattatttctggaaaacgcctcgcaaaaacaaaacataaaatccgctttttaaatgattttccggcgccattttcgcgccacattaatgagtaatataatgagtattagtaatgtgtgtatgcggttttcttcatttacatcgaagaaccgttaaacggctgaacaagcttcggggctggcgtaaggtttctgatcaatttacgcgaagcggtagagcaatatctggaacgtcagcaattcccgaatacgtaaaacaaaggagagcaggcaaaagggaggtagttggtgttgatgatcgttaggagcataagggaatgacaagaattttgttcttgaatataaaaacagatgcccttattctggtattaatgaggctgtttgcgaacttataataactgcaactgttacatcatatctggaaacgcctcgcaaataaaaatgatgcaataaatagagctttcttcaagattcggcaaggtacttttctctccatgtggattcaaaatgatattggcggtgttatgaactctctggcagtacagatatgggcgggaattttactcgatttatcgaatggggtgattcaaagcaacttgatgatctcgaaggtgcagcgcaatgtttcctcgtgcggacctattaagggaagcggtagatcatacctgataatcaaatcaaacaagcaagaaccaatgttcctggcatctggcaaggaaggtgcagaagatgattatcgaatatcggcgtaagctgcgcgagaatggtgtgggaaaatgatgtcaatcagattgctgacaacgtgcccgttgttcgaaatgccggatgcggcgtgaacgccttatccggcctacaaagtcagtataaattcaatgtattgcagtttattggtaggcctgatggctggcgcatcaggcaatcttgctgtcatcggtctcatgcccataaccttattgatgtgggtggtgggtaaattggtaaaccggcactggcggcatggcggtgttaacgcggaatacgagatggtgtcgtcaccacctaacgagctgtaatccgggcgacctgcgccaccggaaaacgtcggggtactcttcacccggaaacaggaacgggttgatggaatgcgaactcttcttcttgtattcgtgcgtccaaagtaccaagaggcgaaggtcatctactacggcttcgttttggtctttttcctgataagaaggtactggtagtgtcgctggtcatcgcagctttctggctttaatgcccggcctatttcgtcatcagcagccagtattacggtttgccgctctctgcggattgctgcattcccgcgcactacgtgccattcagtttcacgggttacggtgcagtaacaccttcggtggtgccaatttgcaccatgctggacttcggcagcagaaccacaaaccgggcaatattgacgttgctcgccaaacattcagcgcgggctttgccggatcaggtcggccatgcgcccggtaggcgacagtgcagccagataaacggcgctttatcgctgctgacggacgagaaaatcaggagcaaacagcgcgctggccatatcttccagctcctgagtcattaccttctccagattctcaatcactgccaccagcgccgggccgctcatttcaggtttcagctcggcaatcagcgccatcaagcagctttccggtgcttatcgcacggcaggcggaatatccagcgggcttgccttgtgcgctggcttctttaatgcgcctgcagtcagatccatctccagcgcacgatttgttcgtacagcaccacttcctgggcggtaaggcgtcagctttgtaaagcgcaggtaatcgcagaggatttattttctgccagctcgcgcagacgctcggcgcggcggttgtataaattcttgagccgaggaacaataacggcggaatcgcatatccaccgtacgtttctcgcgaacccagctcatcttgcggattatgcgaatattcagctctttccgttgtcttgcagttccgcattttctgctgccgggtgatgtttcttcgccctggcattgtatccttccaccatggcattgtcgtgcctttcacccaagggtgaatgccaccatgataaccctgaataacgccacctgcggcaaatagatgcaacacgtgctgtagaatcggatcaccggattgaaagcaaggcgcaaaataaggacgccagataatcacgcgctcgcagcagcagaaccgggaaaataatcgcaccgcccgaagaaacgcatttcggccgaagttataacgcccgtatactcacctcctcgttgacgacgatcttacgaatattcttcttcaaaagatagcatcatccccgattgattggttgtgatgcccagtaacggaaaaacggtgatgaaccctgagacaaaacataaaccacgcaccgacaaacgggtgcagaattctacatatacagctgcgaataccgcggttgcatcaaccagttgaaggacggggcaaaagccgctcaccgccgccggggatgaagcggccacggtgatccagtggttgatacgttccagcgcggtgcagcgcacggtggtgtcgtcgtttcatttgcgctctcgtcttctcttcgtgcagattattctcttcctcatcaccacggttcaggccgacaccccatagtagaagatactggccgcaagggccagccgcaaaataacagccgcgagcggtttcagatgcctttcagaatttgcggtttcttcccggttcgggttctccggcaaaccatgatactgaatttggcttgtcaacgtggtgcaacacattacgtgtactaccgacataccggatcgtacagacccacattgtcgtaaccaccaggttttcagctcagcaacgcgctcgctctttccaacgttttcatcaaactcgtacaagtgaatccgcgcccgttgggcaggtcttcacctgagctgaagttctaccaaccaccgcacggatcgacgcagcgtacattggcgaacacggttgtcagcgcaggtttgagcgcggggtaatgaacggacagcctggtacatgccaccaaccaatgcactgctcggctgaagtcgacattaccgttgacacctgaataattgcacgctacaccaggcacgccttcaggcagcctggatggaacagtacgccacagccgtctttgcggatcaaagccattcagtttgtctggctgtccacttcgagcgcattaccgtccacgatttggcgctaaatcattggggttgtcgtacaccccaatgttattgccgacattgtatcgcagtgtcgttccctctgaacacgccaccacaaccgggctttacagccgatacaggtggtaacgtcgatgagtttcgcccacttcttcctggaagtcccgcgcctgaggcgcggggtcgaacattagtcgcggaacgacgaataagttaaacatgacagacgccgagatagagcgacgagcaaagtaaggaaccccgcctctctgacttggaacctcgttccagcagtacagccaacttg

SEQ ID NO: 11 - DNA, 11605 bp, Artificial Sequence
  Basecall_Alignment_template 90e5fe72_read_ch2_file11
cactttgataagaggttccaagtcattcctactgcctgtcgctctatcttcggcgtctgcttggtgtttaacctattcgtcgttccgcgactaacggtctgaccccgcgcctccaggcgcggaacttcagaaaagtggcgaaactcatcgacgttaccaccagctctggctgtaaacccctgtcaaaggtggcgtgttcaagtggaacgacattcgcgaccgtcgtaataacattggggtgtacgacaaccccaatgatttaaacgcaccaaatcgtggacggtaatgcgcgctatcggtgaacagaacgacaaactggaatggctgatccaccaagacggcagcgtactgttcgatcaggctgcctgggcgtgccggcggaagattaccagtgtcagtatggcctcgtcgacttcagtcccaggcggtgcggtggcatgcggattgtgcgacaccgcgggctgtccgttcgacattccgcgcggaagacaaccgcgtctacaatgtgccgctgtgcgtcgaccgcgtggtggttgggcgaaccagcctgcgtgaagaccaccgcgcgggcgcgattcacttcggtacgaaagagtcggtaaacgctggcgaaacgagcgttgctgagctgaaaacccgcggttacgacaatgcgggtctgtacgatccagcgagaacgtcggtggtacgtcatgtacacgtgccgcaccatgctgaaactgaccaaatctgtatcgcgaagcacaggagactaatcagcgaaaccgcaattctggaaggcctcctggaagccgctcgcggctgttggcttgcggctacccttgcggccagtatgtcccgccgtggtgtcggtcgaaccgtgcggatgagaagaaataatcctgcacgagaaagacgggcgcaaatgaacgacgtgacctgtcgtgcgctactgcgcgccggaacgctatccaaccactggatcaccgccttcttcatcctggcggcggtgagcgggctgggctttatttcccgtcccttcaactggttgatccaccaaatcgccatttaccgcaactggcgttctgcacccgtttgtcagcgtggttcatttgcctcgttcatcatcatgttttccgttgccagcatctggcttcatcaatcgggtaatcttttggcgaagaatattcgtagatcgtcgtcaacgaagtaggtgacaccgggcgttataactggtcagaaatgcgttttcctgggcggcgattatttttctggttctgctgctggtgagcggcgtgattatcagcgatcatatttacgcctgctttctccgtagtgatcgattcgcgttaatgctgccattcatttaccagtggcgacagccagcggattatcatggtgcatatctgcgccgccctttgggtgaaaggcacgatgccgccatgaaggatgtaccagcgcctgtgggcgaaacatcgcacccgcgctgatgccgtgaggtccgcaagacaacggaaagccaatcagtattcgcataatcctggaatgagctgggtcaagcggcttgtacggcgagatatgattccgccgttattgttcctcggctcaaaattaaccgcgccgagctgtctgcgcgagctggcgaaataatcctctggtgattacctgcgctttgctgcgcttatcgcccgccaggaaagtggtgctgtacgaccatccactggagatggtctgtgcgcgcataaaagccagcgcacaaggcaagcccgcagatattcacgttctgccgcgtgataagcactggcaaaaactgctgatggcgctgattgctggcgctgaaaccacaaataggcccggcgctggcggtgaagtctggaggcatcgactcagggctggaagaccagcccagcgcctcctgatttctcgtccgcgtccgtgctgataaaacgccgttgtatcctgggctacgcaatcgctctactggctgaatggccaatctcagtcaacaaagcccgcgctgagccacgacgagcaacgtcagccttgcccggtttgtggtttatgccggtgtccaaagcataagttaccgtggcaccactcggaactacgacctgcactgcaactattgtgaaactgaatagcacgtggtgcgcagccatcaacaactgcgagcaggcgacaaacccattaccattcgctggatgacgagcaaacgcgataaagccaaagctgcgtgacgacgcctgaaaattctctatcggaaaagtccagaaatcaagccgtaacgggtggcctcctctggtactggacgcacgaatgggcaagaggctatgcccgcagttccatcaaccgttcacatttccgggtgaaggtaatctcccgacgttttcgggtaacaggtcgcccggattacagcgctcatggggtgtgacgacaccatctctcgtattcgttaccacctcaaactgtgccgccggtgccagtttgactcaatttcaccacatcaataaggaccttggcggggcggtgacaagcgtagattgcctgatgcgctgcgcgcttatcaggcctaccaataaactgcaatacgatgaatttatacgactttggcaaggccagatggcgttcgccgcatccggcatgaacaacgcgttgtcagcaactcgattgacatcattttattgttcctcgcgcaaccccacgctgatattcgacaccatcttcacaccgcctgccagatgccgggaacactggttcttgctgttgcgttgatttatggtgatgatccagcttccttaatgggtccgcacggaagattacatttgcctcgagatcatcgttgtaatcacctcattcgtcgtcaggtaaaattctgcccatatctatacctgccaaagttcaccaatatcacttcaatatcattttgaatctggaaaagtaccctgccgaatctttaaaaactcatttacacttatcattttattttgcgaggcgttttcagatatggtcatggcagttgcggattatattcaagtaaaacaaccttgtattaataccagaataagggcatctgtactatgttcaaaattgaaaattttgtcattccttatgctcttacactgatcatcataccaactacctccccctttgcctgctccttacagcactgggaattactgacgttcagatattgctctaccacttcgcatccattgcagatcgtgaaacccacgccagcaagcgttccgtgttagtgcctcttctgataaatgaaaaaccgtatacatcgccattaataccttgtattactcagccaatgctgtgcgaaagtatggaaaatcatttaagcggattttgcatgttgttttgttgcgaggcgttttccatatgctctatagagtgttgcgttgtttcatttattactcaaatggttagttatcgctaaagtggattatgattactatgaatatattatattcagaatgttgttgcataatctgaatggtgtaactgaaaaacatatcagcatcctaacagcaccggattttaaattgaaattaatctttcatctgaaccggtcagtactgccgcaaccggtctttacttgctctatattctatatttgtggtaatgattcaggaaggattgttttctaaattaacaacagaataactttcttgtttaatgagattaatgtggcaaccattataataccacggtttagagcaaacatacaacatattattcataacatacagagcagtaaatgaatgatactgacaatgatgctagtccattatctttgcataatatttattgctataatttaaaaatatttatgagaaagtatggcacagagaacgactatcaagtatcagcaaactaagatgatggtggcattatctgcgataaaattgccactcagttctacaaataatatttaaatatactgaacagtgatctgtgaacgtaagacccaacgagaataaaaatttatagagttcttgttttaatataacgaaaccgggaccagcaaatgacctgaatagggagaacgcttgcctatgccatcagctactcttcttcgttcctcctcttcttaccgggccaaatagctgcgccaggcgaacgatacgtgccttcaaacagctgcacccggcgtctcgtcgccaagattttcgacctgcatctgccgcggccagcgccgtcgcgcgccagacggtcgagatcgccgctgagcaccgaggtcggctaccgcatgagtttaccgctatcggccttggcggcggttaagccgcatcccatcacgaacaagtcgttccgccggggtgtggcgaccgcagcatcggccagataagtcccaaccagtgagcgtcgccagtgaataaactcccgaaacaaaaccgccgtatggtgcagttcctgattacggttctggcatggtagtgaccgtacgcccggtatgatacccgaatgcgcgccattttcactggcgcggaatatgttcgtaccacgcctgttcgctgcgcgcaccgccgcgatgcggtcatccagagtggcgacgggcttaatcgtggcgaatcggcgtgtggttggcgtggtgatttctcccagtgctcggcaacggcgaaaaactcaccgcgtcttcacgggcgctacaggtcgcacgccaacgccttcctgacgccaccgactccaggtcatcgccatcggcgcccttcatcctgcgtcgggatgaacggccataaagcaaatggacgcttcattgtcggcattaatatacggcctaccgccagattaccctgctcgtcgacgaccatctggtgatgcgccatcgcatcccacgcgtcgcgttcagaaccttttggttgatgcgagcacgacatttcagcagagcctgataacgcatacaattcttcctgcacggaaccgaaggtgatacgccagcgtactctcttgtttcccgtgacgaccctgaaacttcagctcgcctgcaaccaagaatgtcacgggccatcgtgataacgataccctgcatatcccgcagcgaagcgtgtttgcgtgttcatctcttgcggcggcggcgttcgacgaaatagtcatataacgcctctgcgcgatccggtgatgcacctttgggcttgggctttgtcccgttcagtatcacggcgagggctgaaaccaccagcctgccgccgcctgttgcgttgagattcatcttgcttcggcatcgctaaaatccggtatgagcacgtgattctcctttcgacacccaataacaaggtccgcgccaatttcgcccgtcgcctatcctctacatttgggattacgcgttaattaatgcaatcatggttcgtcattcttgttcttcttgctggttgcggtattccccgagtggtaatttcgcgccaagcagacgtacaccatgtcagtgttaaaacgaagagaatggtcaccgccagcacaccataaatgagctgatatgagcggaacatgatgtaaacgcaaacctttcttctgctgattaagtgcggcgacaaaacgcgccaaacgataaatcgcggttaggtacgccggatggtaggaacaatgctgtacagcaaccagagatccccgacaacaggaaaaatacgcagcacgttgtcggtaaccgtattgatcctcgccagcgcaggagaaggcaatgaactgatcgccagactggcccctaccagcattcgcaaatcatccagtacgaacagtaaattttggtcgcgctcgtttaccacgccagatggtattcaacgctatcgatggagtacatcagcaacaataacgcggtgacgtcagcccgcacgccccaacggcggtcatcttgttgggtggcaacaaattgttcgatataccgctggtaacatcgccagtagcaggcgaagttgcttaaagtagtgacggcttgaatgctgacgtcgaaaacatgggaaaagcgacgctttaaaagcaacggcagccagcggcactaatgaacaacgacccttgagcaaggttacctgccagggttgtcatgttgtcctctcaatgcgttggtagtttgctttcgaccttggacgggtacggtgcctggctttgtctgaatggttttaacaacactagcgaaacggtccgggatcaggtggttgctcgctactgatgctggtaatgcccggctgattggctccttctatgacccatcggcgttatcgtcgaaagaccttatcgctgggtgaaaacgccttccgccgcaaacatgctgttaattcagccttttcgggacgcatctagatcttgcgacagatagatatgattgtagcatcacaattttccgggtattctccggcagaaggtggtatgcgagcggttgtggaagcaccacccgcatgatacctgctcacgcagtttgtgcatgatgtggcgatcacttccgggcgcagcgcagcaaacaccgcctgccagccgtgagagagcgctgctcgtagcttggctgagccaaatctcgtgacacagcgcctctgcgaacgcttcgtcataatttccccacactcatgctgatgaaacactaccatatgaaaactcttcttaagcgatgccagcggaatacgcgttgaaatcatcaggctcccaacacggttaaagtcgatatcgacaacattacctaaatcaagatatagagcattttgcctcctttcgcgccacaagaagtgctgtagcaggaaaggatgggtttaactatgtggcaagtgtaaaccaggttaacggtcacaaaatctacgcgtcttcctgggaaaatgatttcgttggctgtctcccaaccgaaaacgtgattttagcgccggcgagcggcaactcgtcggtaagagcgcagtgacctgtgccacgttaccaatttcaaaaacctgccaagcatgatgccgtgtgatcggcgaccagcagggctgttctcgcgtacgccatcatgtttcaccacgccgctgaacacatcaactccatcaacgcgccatcctctaatcgctaaccttacattcaataatcggcacaatcatacaaaggacgcgctgaagggccaatgatcccgctattatgaggcgcaacgtaccgccgggcactatcgctttaaacgcgggttgcggtaaagaataatgcgccgcgcaggcttcggtggtgattatccgcaaatgattatggttcgtaacgcggcaacatgctcaacagtcatgccaatggtgataatattgttgaatataagacctggtctgccaccgctgcggcaatcgctttttctcggtttgcgaaacctcgctgctcgaacgccgtattaacgacactggaagcccgacccgcgccaccgtgatggcgcgtaatcagaactgccgctcatggtgaatatccccagcggaccgtctgcgtggagacatccaacgaatttgccaacaatatcataaatataccacgctcgacacgatcaacactggtggtcgtgccgcgggttaccggttagttcagtgggctgtgaaaaattcctcgaaaaccatcaccctggcattttgccaaaaggtgacaaaaagatcgggtttgatcggtcactggggatcccgaagcaaatcccgccggatgatgtcgtttgcccgctacccgctggcgaagcggactgactcgcttcatcccaccacttgttgccagcgccaccgccaaagcgccgtgaaaacatcacccgcagtacatcaccaccacctcggctttgaaggccggttgatgctggcgcccaccaccagtagtcgcagcctgcacgctaccctgggtcataggcatgacaaatttagccaggcgacatgcctgttttggcgctgtctcttttcgcccgttaagcgcgccagacccggttctgaggccgcgcgatcgcgaaacgctactacccggctcacgccgatatcctgcggcgtaatccccgtccagaacaggtcatcaccgcctgacggtggggtgaagaacttttagcgccgtctgccagcgtacgtctgccagcacaacatcccgcaggaaatcgatttcctcaaccgcctctgcatcatcaggcagcagatccgggctggggtggttaatgattatccgctctgctagcggtatccgcatgatggccggattgccgaagatttcgcctggttataccgtttggtgtaacgggtgttaacgcccaggattccagctctgccagcaggctgttgccgatgtctgtcatcacctacgtatgcatcgaccctgcgcccacaacctttacccgccaccaaccgctaccgtcgccgctggcctgcaacttccgtataatttctcgccacatgcccaccgctctcgtcgtgtccttccacgtaatagatgcgatcctgtccacgtttatacctacacaagcagatcatggtcattctccttaaacattgcgggatgcgttcattttaattcaccagtgtttaaaagtgacggctacatcaattttgactgtcgatacaaaccagtcaaacgaacaaagcaaagcatgtcataaatgacaaaaagtgacataactgtattcaggagggttatggcaacaatcaccgacctcgttttacggacaatgggtccgccaatggcgagcaatttattgcagcaagaacgtaacttcgcgtcttgatgtgaacgccgaagctgccgacatctggtgaacaaggtgcgactcgccgccaaccggcgcagaccactaaagatgaatttatcattactgttcttgaatggcgatctggtgcgcaacattgttctgattgaaaacggcgtttgcgaaggcttatctgttcgctggtcgttgatatgtccacctcatgcaaaccgataaattcgttgccgatatacagcaaaggcttcagcatgatggatgttccgacgaaaccgtacttctgcaaatgccattaccggtactctgttactgctgatggcggcctgaaccgttgaacgatgccacgcccgtcccaccggtggcgatgggcggtggttgatcgcgctggcggtccgggcatggggatcacgttagctcatcagcaactacatgagcatcgcgctcaatgcgctctgacggaaaccgccgtttgtgaccctggatcttccgtgttgccgcaaagtgatgagcgcacgccgcaagtaagatcttcaccgcttcggcaaacaagtctcggcggagatcttctccgccatactcatgatcgatcttgccgcagaatcccagcatcgccttgatgtcgccaaccaaagctgcatcgtgccaatgctggggccgcctcgcagggttgtaactgagcgcgcggcgatcgcgatcgccaggacggtccgccattctggagcaggtcgtgtcaggtctgggatggctaccagtaaaaatgtaacgactggataaaggaataaatgaatgaataagtacaccatcaacgacattacgcgcgcatcgggcggttttgccatactggcggtcgatcagcaagccatgccgcaatgtttaccacagctggggcacctgctcggtagccgtgggcacaacgatttcaaagttaacactgcaaggccctctcgccttgtcctcggcgattctggtagatcagcaattcgccaccgccaggtggttgagcaaacgcgttatagcaggacgcgccatgattgtcatgccgatgagttcattctacagcagcagtattccggtcgatagcatggtgtcgaccgcaaaatcaatcgctacagatcaaacaagacggtggcaagcggcaaaactgctggtgctgtggcgtgatgaagatgcgcagcagcgtctggatatggtgaagagttcggcgaactgtgccactcacacggtgttgagccagtcattccgcccaccgcgtcgtggcgataaattcgatcgcgaacaagcgatcatcgataccgccagagctgggcgacggtggcgctgacctctcaaagttgaaatgccgctttatggcaggtccgcaacagaacttctgcttcacaacgtcagaccgagccacatcaatatgccatgcgggtgatctctcttccggtgtctcgtaagctgttcccgcattgccgtacgcgtggcaatgacggcgggcgcatcggacctggcaggccgtgcggtctgggcatcggtcgtcggtttaccagacaacgagctgatgctgcgtgacgtttgcaccgaagtacaacaacagcgacatcgtcagcaaaccaatggctaaacgccgctatgaatgaggataaagatggtttaacacctaagcttacaaccgttggctggaacggaaaccgaccatctttgattttggtaaaaattccgtagtgccgactggtttggctggttaggcaataaaggcaaatcaaagagatgggcaccatctgtggatcaccgctcattgcgtttattccgttgccacggcgtgggtcgacctggcgcttactcgttggttgatcacggtatcaagccatgagcgtgataaatatggcggctgagccatgcctgcacgtgaatgacggggcgtggtggatgcctcgagcagatatcaacgctaacagcatgccagcacgggtgcctgccagcgccgtcacggcagattttccaggcgctcgttacaccattgaaattatccagaaatatttctgaacgaagaaggcagatgtgctggagtcctgggacgaagccttccagcaaaaccgaagagtaccgcgacggcaatgccatatgcacgcggtggaaacttctcttgattgtttatgacgtcactcacgacaaaaatgagctggatcgcgcgattcgcgtggcttccccgcgatatccggcaatcgccgaaataatcattatcgcgttaacgaacacttcgatacccgtggaatccgctgccggattacaacaaagatcgccggcacgtcgcttccgcgcgttcgggtacaccaggccactggatcgaatggggccgtttaatgctgcacatcatgctgcctggaagcccgttgcgaacaaccagcgtaacgctgaagataccaaggtctgtttaacgccaccgtgcgcgatgcctgggcacccgatggcgcggacgggattgcgacataccgttgactgggaaggaaaaccggtggtccgcgaacgatgtacgttggcctatcaagcaatggtacggcctacgcgctccaccgtcactggcgatcgccagtatgaaaccctggtatcaaacatggtggggtgcattgagtacctgatggactatgaaaatggttcctggtggcggagctggatgcagttaatggtcctacaaagtctgggacgctaaacaggatattatcacctgctgcattgcctgagtgatcccacgtatcccgttagcgcccggcatgctccagcagtttgcagcagattactggataataatgcgaaataactgatctgaaaataggtgcgggtttcctctaaccctctccccaaaggggcgaggggacgtccggtgcagaaggttaaacgcaagcagacgccgaagatagagcattgagcaaggaacactctcgtttggaacatctggcaaacgcgaagcagacgccagcaatacgtaac

SEQ ID NO: 12 - DNA, 61 bp, Artificial Sequence
  Adapter design A/B (top strand)
  misc_binding (1)..(1): nucleotides preceded by 1x 5SpC3 and 29x iSpC3
  misc_binding (33)..(34): nucleotides separated by 1x iSp18
ggcgtctgcttgggtgtttaaccttttttttttaatgtacttcgttcagttacgtattgct

SEQ ID NO: 13 - DNA, 40 bp, Artificial Sequence
  Adapter design A (blocker strand)
  modified_base (1)..(1): 5BNA-G
  modified_base (2)..(2): iBNA-G
  modified_base (3)..(3): iBNA-T
  modified_base (4)..(4): iBNA-T
  modified_base (5)..(5): iBNA-A
ggttaaacacccaagcagacgcctaagtcagagaggttcc

SEQ ID NO: 14 - DNA, 45 bp, Artificial Sequence
  Adapter design A (bottom strand)
  modified_base (23)..(23): iBNA-A
  modified_base (24)..(24): iBNA-meC
  modified_base (25)..(25): iBNA-A
  modified_base (26)..(26): iBNA-T
  modified_base (27)..(27): iBNA-T
gcaatacgtaactgaacgaagtacatttttgaggcgagcggtcaa

SEQ ID NO: 15 - DNA, 41 bp, Artificial Sequence
  Adapter design B (blocker strand)
ggttaaacacccaagcagacgcctttgaggcgagcggtcaa

SEQ ID NO: 16 - DNA, 47 bp, Artificial Sequence
  Adapter design B (bottom strand)
  modified_base (23)..(23): iBNA-A
  modified_base (24)..(24): iBNA-meC
  modified_base (25)..(25): iBNA-A
  modified_base (26)..(26): iBNA-T
  modified_base (27)..(27): iBNA-T
gcaatacgtaactgaacgaagtacattttttaagtcagagaggttcc

SEQ ID NO: 17 - DNA, 80 bp, Artificial Sequence
  follow-on adapter top strand
  misc_binding (44)..(45): nucleotides separated by 4x iSp18
taacgaggttgtttctatctcggcgtctgcttgggtgtttaacctttttgtcagagaggttccaagtcagagaggttcct

SEQ ID NO: 18 - DNA, 123 bp, Artificial Sequence
  follow-on adapter bottom strand
  misc_binding (35)..(36): nucletoides separated by 4x iSp18
  misc_binding (98)..(99): nucletoides separated by 4x iSp18
ggaacctctctgacttggaacctctctgacaaaaaggttaaacacccaagcagacgccgagatagaaacaacccatcagattgtgtttgttagtcgctagcgactaacaaacacaatctgatg

SEQ ID NO: 19 - DNA, 70 bp, Artificial Sequence
  concatenation sequencing adapter top strand
  misc_binding (15)..(16): nucleotides separated by 15x iSpC3
  misc_binding (48)..(49): nucleotides separated by 1x iSp18
ggttgtttctatctcggcgtctgcttgggtgtttaaccttttttttttaatgtacttcgttcagttacgt

SEQ ID NO: 20 - DNA, 41 bp, Artificial Sequence; identical to SEQ ID NO: 15
  concatenation sequencing adapter blocker strand

SEQ ID NO: 21 - DNA, 28 bp, Artificial Sequence
  concatenation sequencing adapter bottom strand
  modified_base (24)..(24): iBNA-A
  modified_base (25)..(25): iBNA-meC
  modified_base (26)..(26): iBNA-A
  modified_base (27)..(27): iBNA-T
  modified_base (28)..(28): iBNA-T
tcgttaacgtaactgaacgaagtacatt

SEQ ID NO: 22 - DNA, 71 bp, Artificial Sequence
  fishing adapter top strand
  misc_binding (1)..(1): nucleotides preceded by 1 x 5SpC3 and 14 x iSpC3
  misc_binding (16)..(17): nucleotides separated by 15 x iSpC3
  misc_binding (49)..(50): nucleotides separated by 1 x iSp18
ttgtcagagaggttccggcgtctgcttgggtgtttaaccttttttttttaatgtacttcgttcagttacgt

SEQ ID NO: 23 - DNA, 22 bp, Artificial Sequence
  fishing adapter bottom strand
  modified_base (18)..(18): iBNA-A
  modified_base (19)..(19): iBNA-meC
  modified_base (20)..(20): iBNA-A
  modified_base (21)..(21): iBNA-T
  modified_base (22)..(22): iBNA-T
acgtaactgaacgaagtacatt

SEQ ID NO: 24 - DNA, 100 bp, Artificial Sequence
  fishing tether top strand
ttgtcagagaggttccttttttttttttttttttttttttttttttttttttttggttgtttctgttggtgctgatattgcttttttgaccgctcgcctc

SEQ ID NO: 25 - DNA, 31 bp, Artificial Sequence
  fishing tether bottom strand
  misc_binding (29)..(30): nucleotides separated by 6x iSp18
gcaatatcagcaccaacagaaacaacctttt

SEQ ID NO: 26 - DNA, 3587 bp, Artificial Sequence
  3.6kb dA-tailed DNA
gccatcagattgtgtttgttagtcgctgccatcagattgtgtttgttagtcgctttttttttttggaattttttttttggaattttttttttgcgctaacaacctcctgccgttttgcccgtgcatatcggtcacgaacaaatctgattactaaacacagtagcctggatttgttctatcagtaatcgaccttattcctaattaaatagagcaaatccccttattgggggtaagacatgaagatgccagaaaaacatgacctgttggccgccattctcgcggcaaaggaacaaggcatcggggcaatccttgcgtttgcaatggcgtaccttcgcggcagatataatggcggtgcgtttacaaaaacagtaatcgacgcaacgatgtgcgccattatcgcctagttcattcgtgaccttctcgacttcgccggactaagtagcaatctcgcttatataacgagcgtgtttatcggctacatcggtactgactcgattggttcgcttatcaaacgcttcgctgctaaaaaagccggagtagaagatggtagaaatcaataatcaacgtaaggcgttcctcgatatgctggcgtggtcggagggaactgataacggacgtcagaaaaccagaaatcatggttatgacgtcattgtaggcggagagctatttactgattactccgatcaccctcgcaaacttgtcacgctaaacccaaaactcaaatcaacaggcgccggacgctaccagcttctttcccgttggtgggatgcctaccgcaagcagcttggcctgaaagacttctctccgaaaagtcaggacgctgtggcattgcagcagattaaggagcgtggcgctttacctatgattgatcgtggtgatatccgtcaggcaatcgaccgttgcagcaatatctgggcttcactgccgggcgctggttatggtcagttcgagcataaggctgacagcctgattgcaaaattcaaagaagcgggcggaacggtcagagagattgatgtatgagcagagtcaccgcgattatctccgctctggttatctgcatcatcgtctgcctgtcatgggctgttaatcattaccgtgataacgccattacctacaaagcccagcgcgacaaaaatgccagagaactgaagctggcgaacgcggcaattactgacatgcagatgcgtcagcgtgatgttgctgcgctcgatgcaaaatacacgaaggagttagctgatgctaaagctgaaaatgatgctctgcgtgatgatgttgccgctggtcgtcgtcggttgcacatcaaagcagtctgtcagtcagtgcgtgaagccaccaccgcctccggcgtggataatgcagcctccccccgactggcagacaccgctgaacgggattatttcaccctcagagagaggctgatcactatgcaaaaacaactggaaggaacccagaagtatattaatgagcagtgcagatagagttgcccatatcgatgggcaactcatgcaattattgtgagcaatacacacgcgcttccagcggagtataaatgcctaaagtaataaaaccgagcaatccatttacgaatgtttgctgggtttctgttttaacaacattttctgcgccgccacaaattttggctgcatcgacagttttcttctgcccaattccagaaacgaagaaatgatgggtgatggtttcctttggtgctactgctgccggtttgttttgaacagtaaacgtctgttgagcacatcctgtaataagcagggccagcgcagtagcgagtagcatttttttcatggtgttattcccgatgctttttgaagttcgcagaatcgtatgtgtagaaaattaaacaaaccctaaacaatgagttgaaatttcatattgttaatatttattaatgtatgtcaggtgcgatgaatcgtcattgtattcccggattaactatgtccacagccctgacggggaacttctctgcgggagtgtccgggaataattaaaacgatgcacacagggtttagcgcgtacacgtattgcattatgccaacgccccggtgctgacacggaagaaaccggacgttatgatttagcgtggaaagatttgtgtagtgttctgaatgctctcagtaaatagtaatgaattatcaaaggtatagtaatatcttttatgttcatggatatttgtaacccatcggaaaactcctgctttagcaagattttccctgtattgctgaaatgtgatttctcttgatttcaacctatcataggacgtttctataagatgcgtgtttcttgagaatttaacatttacaacctttttaagtccttttattaacacggtgttatcgttttctaacacgatgtgaatattatctgtggctagatagtaaatataatgtgagacgttgtgacgttttagttcagaataaaacaattcacagtctaaatcttttcgcacttgatcgaatatttctttaaaaatggcaacctgagccattggtaaaaccttccatgtgatacgagggcgcgtagtttgcattatcgtttttatcgtttcaatctggtctgacctccttgtgttttgttgatgatttatgtcaaatattaggaatgttttcacttaatagtattggttgcgtaacaaagtgcggtcctgctggcattctggagggaaatacaaccgacagatgtatgtaaggccaacgtgctcaaatcttcatacagaaagatttgaagtaatattttaaccgctagatgaagagcaagcgcatggagcgacaaaatgaataaagaacaatctgctgatgatccctccgtggatctgattcgtgtaaaaaatatgcttaatagcaccatttctatgagttaccctgatgttgtaattgcatgtatagaacataaggtgtctctggaagcattcagagcaattgaggcagcgttggtgaagcacgataataatatgaaggattattccctggtggttgactgatcaccataactgctaatcattcaaactatttagtctgtgacagagccaacacgcagtctgtcactgtcaggaaagtggtaaaactgcaactcaattactgcaatgccctcgtaattaagtgaatttacaatatcgtcctgttcggagggaagaacgcgggatgttcattcttcatcacttttaattgatgtatatgctctcttttctgacgttagtctccgacggcaggcttcaatgacccaggctgagaaattcccggaccctttttgctcaagagcgatgttaatttgttcaatcatttggttaggaaagcggatgttgcgggttgttgttctgcgggttctgttcttcgttgacatgaggttgccccgtattcagtgtcgctgatttgtattgtctgaagttgtttttacgttaagttgatgcagatcaattaatacgatacctgcgtcataattgattatttgacgtggtttgatggcctccacgcacgttgtgatatgtagatgataatcattatcactttacgggtcctttccggtgaaaaaaaaggtaccaaaaaaaacatcgtcgtgagtagtgaaccgtaagc

SEQ ID NO: 27 - DNA, 41 bp, Artificial Sequence
  follow-on adapter bottom strand
acgtaactgaacgaagtacatttttgaggccgagcggtcaa

SEQ ID NO: 28 - DNA, 40 bp, Artificial Sequence; identical to SEQ ID NO: 13
  follow-on adapter blocker strand

SEQ ID NO: 29 - DNA, 38 bp, Artificial Sequence
  FO016_FOSEN_tailattach_TOP_A
ggtgctgaagaaagttgtcggtgtctttgtgttaacct

SEQ ID NO: 30 - DNA, 60 bp, Artificial Sequence
  FO017_FOSEN_tailattach_BOT_A
ggttaacacaaagacaccgacaactttcttcagcaccagcaattaagtcagagaggttcc

SEQ ID NO: 31 - DNA, 77 bp, Artificial Sequence
  FO018_FOSEN_tailattach_TOP_B
  misc_binding (23)..(24): nucleotides separated by 4x iSp18
ccaatttgtgggttcgtctgcggtttttggcgtctgcttgggtgtttaaccaaggcgtctgcttgggtgtttaacct

SEQ ID NO: 32 - DNA, 99 bp, Artificial Sequence
  FO019_FOSEN_tailattach_BOT_B
  misc_binding (53)..(54): nucleotides separated by iSp18
ggttaaacacccaagcagacgccttggttaaacacccaagcagacgccaaaaaccgcagacgaacccacaaattggagcaattaagtcagagaggttcc

SEQ ID NO: 33 - DNA, 82 bp, Artificial Sequence
  FO020_FOSEN_tailattach_BOT_B_noside
  misc_binding (53)..(54): nucleotides separated by 4x iSp18
ggttaaacacccaagcagacgccttggttaaacacccaagcagacgccaaaaaccgcagacgaacccacaaattggagcaat

SEQ ID NO: 34 - DNA, 66 bp, Artificial Sequence
  FO021_FOSEN_tailattach_TOP_C
  misc_binding (23)..(24): nucleotides separated by 4x iSp18
ggcgtctgcttgggtgtttaacctttttggtgctgaagaaagttgtcggtgtctttgtgttaacct

SEQ ID NO: 35 - DNA, 88 bp, Artificial Sequence
  FO022_FOSEN_tailattach_BOT_C
  misc_binding (42)..(43): nucleotides separated by 4x iSp18
ggttaacacaaagacaccgacaactttcttcagcaccaaaaaggttaaacacccaagcagacgccagcaattaagtcagagaggttcc

SEQ ID NO: 36 - DNA, 44 bp, Artificial Sequence
  FO023_FOSEN_splintagain_TOP_A
  misc_binding (15)..(16): nucleotides separated by 4x iSp18
ccaatttgtggttcctttttggcgtctgcttgggtgtttaacct

SEQ ID NO: 37 - DNA, 49 bp, Artificial Sequence
  FO024_FOSEN_splintagain_BOT_A
  misc_binding (28)..(29): nucleotides separated by 4x iSp18
ggttaaacacccaagcagacgccaaaaaggaaccacaaattggagcaat

SEQ ID NO: 38 - DNA, 69 bp, Artificial Sequence
  FO025_FOSEN_splintagain_TOP_B
  misc_binding (15)..(16): nucleotides separated by 4x iSp18
ccaatttgtggttcctttttggcgtctgcttgggtgtttaaccaaggcgtctgcttgggtgtttaacct

SEQ ID NO: 39 - DNA, 74 bp, Artificial Sequence
  FO026_FOSEN_splintagain_BOT_B
  misc_binding (53)..(54): nucleotides separeted by 4x iSp18
ggttaaacacccaagcagacgccttggttaaacacccaagcagacgccaaaaaggaaccacaaattggagcaat

SEQ ID NO: 40 - DNA, 61 bp, Artificial Sequence
  FO027_TOP_1sp18
  misc_binding (23)..(24): nucleotides separated by 1x iSp18
ggcgtctgcttgggtgtttaacctttttgtcagagaggttccaagtcagagaggttccaat

SEQ ID NO: 41 - DNA, 66 bp, Artificial Sequence
  FO028_BOT_1sp18
  misc_binding (37)..(38): nucleotides separated by 1x iSp18
ttggaacctctctgacttggaacctctctgacaaaaaggttaaacacccaagcagacgccagcaat

SEQ ID NO: 42 - DNA, 45 bp, Artificial Sequence
  FO029_TOP_1hybsite
  misc_binding (23)..(24): nucleotides separated by 4x iSp18
ggcgtctgcttgggtgtttaacctttttgtcagagaggttccaat

SEQ ID NO: 43 - DNA, 50 bp, Artificial Sequence
  FO030_BOT_1hybsite
  misc_binding (21)..(22): nucleotides separated by 4x iSp18
ttggaacctctctgacaaaaaggttaaacacccaagcagacgccagcaat

SEQ ID NO: 44 - DNA, 40 bp, Artificial Sequence; identical to SEQ ID NO: 13
  Blocker strand ID2 (TT008)

SEQ ID NO: 45 - DNA, 14 bp, Artificial Sequence
  Pore-tether
ggaacctctctgac

SEQ ID NO: 46 - DNA, 47 bp, Artificial Sequence; identical to SEQ ID NO: 16
  Bottom strand ID5 (TT186)

SEQ ID NO: 47 - DNA, 59 bp, Artificial Sequence; identical to SEQ ID NO: 3
  FO003 duplex stem example top

SEQ ID NO: 48 - DNA, 64 bp, Artificial Sequence; identical to SEQ ID NO: 4
  FO004_Duplex stem example bot

SEQ ID NO: 49 - DNA, 44 bp, Artificial Sequence
  Barcode 1nt overhang
gcaatacgtaacgtaacgaagtacatttaagtcagagaggttcc

SEQ ID NO: 50 - DNA, 39 bp, Artificial Sequence
  Barcode 6nt overhang
acgtaacgtaacgaagtacatttaagtcagagaggttcc

SEQ ID NO: 51 - protein, 439 aa, enterobacteria phage T4
MTFDDLTEGQKNAFNIVMKAIKEKKHHVTINGPAGTGKTTLTKFIIEALISTGETGIILAAPTHAAKKILSKLSGKEASTIHSILKINPVTYEENVLFEQKEVPDLAKCRVLICDEVSMYDRKLFKILLSTIPPWCTIIGIGDNKQIRPVDPGENTAYISPFFTHKDFYQCELTEVKRSNAPIIDVATDVRNGKWIYDKVVDGHGVRGFTGDTALRDFMVNYFSIVKSLDDLFENRVMAFTNKSVDKLNSIIRKKIFETDKDFIVGEIIVMQEPLFKTYKIDGKPVSEIIFNNGQLVRIIEAEYTSTFVKARGVPGEYLIRHWDLTVETYGDDEYYREKIKIISSDEELYKFNLFLGKTAETYKNWNKGGKAPWSDFWDAKSQFSKVKALPASTFHKAQGMSVDRAFIYTPCIHYADVELAQQLLYVGVTRGRYDVFYV

SEQ ID NO: 52 - DNA, 69 bp, Artificial Sequence; identical to SEQ ID NO: 38
  adapter top strand

SEQ ID NO: 53 - DNA, 74 bp, Artificial Sequence; identical to SEQ ID NO: 39
  adapter bottom strand